European Patent Application EP 4 509 144 A1, published February 19, 2025. Title: APTAMER, CONJUGATE, COMPOSITION, METHOD FOR PREPARING SAME, AND USE THEREOF. Applicant: SUZHOU RIBO LIFE SCIENCE CO., LTD. The sequence listing filed with the application follows.

SEQUENCE LISTING (82 sequences)

SEQ ID NO: 1 - RNA, 21 nt, synthetic construct
  source 1..21: mol_type = other RNA
ctgcttcagacgtgttagctt

SEQ ID NO: 2 - RNA, 22 nt, synthetic construct
  source 1..22: mol_type = other RNA
ctgagttcagacgtgttgctct

SEQ ID NO: 3 - RNA, 32 nt, synthetic construct
  source 1..32: mol_type = other RNA
tctatggctgccgatctggtctccatgtacgt

SEQ ID NO: 4 - RNA, 21 nt, synthetic construct
  source 1..21: mol_type = other RNA
  misc_feature 1: note = is CT, TC or AC
  misc_feature 13: note = is T, C or G; or a motif consisting of two of T, C or G
  misc_feature 16: note = is T, CT or TT
  misc_feature 21: note = is T, TT, or TTX, wherein X is a motif consisting of 1-15 nucleotides
nggagttcannnntgngctcn

SEQ ID NO: 5 - RNA, 24 nt, synthetic construct
  source 1..24: mol_type = other RNA
ctggagttcagacgtgttgctctt

SEQ ID NO: 6 - RNA, 24 nt, synthetic construct
  source 1..24: mol_type = other RNA
ctggagttcagacgttgtgctctt

SEQ ID NO: 7 - RNA, 24 nt, synthetic construct
  source 1..24: mol_type = other RNA
ctggagttcagaccgtgtgctctt

SEQ ID NO: 8 - RNA, 23 nt, synthetic construct
  source 1..23: mol_type = other RNA
ctggagttcagacgtgttgctct

SEQ ID NO: 9 - RNA, 24 nt, synthetic construct
  source 1..24: mol_type = other RNA
acggagttcagacgtgttgctctt

SEQ ID NO: 10 - RNA, 24 nt, synthetic construct
  source 1..24: mol_type = other RNA
ctggagttcactactgttgctctt

SEQ ID NO: 11 - RNA, 24 nt, synthetic construct
  source 1..24: mol_type = other RNA
ctggagttcagttgtgttgctctt

SEQ ID NO: 12 - RNA, 32 nt, synthetic construct
  source 1..32: mol_type = other RNA
ctggagttcagacgtgttgctcttccgatctc

SEQ ID NO: 13 - RNA, 32 nt, synthetic construct
  source 1..32: mol_type = other RNA
ctggagttcagacgttgtgctcttccgatctc

SEQ ID NO: 14 - RNA, 32 nt, synthetic construct
  source 1..32: mol_type = other RNA
ctggagttcagaccgtgtgctcttccgatctc

SEQ ID NO: 15 - RNA, 32 nt, synthetic construct; identical to SEQ ID NO: 12
  source 1..32: mol_type = other RNA

SEQ ID NO: 16 - RNA, 24 nt, synthetic construct
  source 1..24: mol_type = other RNA
ctggagttcagacgtgttgctctt

SEQ ID NO: 17 - RNA, 32 nt, synthetic construct; identical to SEQ ID NO: 13
  source 1..32: mol_type = other RNA

SEQ ID NO: 18 - RNA, 24 nt, synthetic construct
  source 1..24: mol_type = other RNA
ctggagttcagacgttgtgctctt

SEQ ID NO: 19 - RNA, 32 nt, synthetic construct; identical to SEQ ID NO: 14
  source 1..32: mol_type = other RNA

SEQ ID NO: 20 - RNA, 24 nt, synthetic construct
  source 1..24: mol_type = other RNA
ctggagttcagaccgtgtgctctt

SEQ ID NO: 21 - RNA, 32 nt, synthetic construct; identical to SEQ ID NO: 12
  source 1..32: mol_type = other RNA

SEQ ID NO: 22 - RNA, 24 nt, synthetic construct
  source 1..24: mol_type = other RNA
ctggagttcagacgtgttgctctt

SEQ ID NO: 23 - RNA, 32 nt, synthetic construct; identical to SEQ ID NO: 13
  source 1..32: mol_type = other RNA

SEQ ID NO: 24 - RNA, 24 nt, synthetic construct
  source 1..24: mol_type = other RNA
ctggagttcagacgttgtgctctt

SEQ ID NO: 25 - RNA, 32 nt, synthetic construct; identical to SEQ ID NO: 14
  source 1..32: mol_type = other RNA

SEQ ID NO: 26 - RNA, 24 nt, synthetic construct
  source 1..24: mol_type = other RNA
ctggagttcagaccgtgtgctctt

SEQ ID NO: 27 - RNA, 23 nt, synthetic construct
  source 1..23: mol_type = other RNA
ctggagttcagacgtgttgctct

SEQ ID NO: 28 - RNA, 22 nt, synthetic construct
  source 1..22: mol_type = other RNA
ctgagttcagacgtgttgctct

SEQ ID NO: 29 - RNA, 21 nt, synthetic construct
  source 1..21: mol_type = other RNA
ctgcttcagacgtgttagctt

SEQ ID NO: 30 - RNA, 24 nt, synthetic construct
  source 1..24: mol_type = other RNA
acggagttcagacgtgttgctctt

SEQ ID NO: 31 - RNA, 24 nt, synthetic construct
  source 1..24: mol_type = other RNA
ctggagttcactactgttgctctt

SEQ ID NO: 32 - RNA, 24 nt, synthetic construct
  source 1..24: mol_type = other RNA
ctggagttcagttgtgttgctctt

SEQ ID NO: 33 - RNA, 32 nt, synthetic construct; identical to SEQ ID NO: 3
  source 1..32: mol_type = other RNA

SEQ ID NO: 34 - RNA, 32 nt, synthetic construct; identical to SEQ ID NO: 12
  source 1..32: mol_type = other RNA

SEQ ID NO: 35 - RNA, 24 nt, synthetic construct
  source 1..24: mol_type = other RNA
ctggagttcagacgtgttgctctt

SEQ ID NO: 36 - RNA, 32 nt, synthetic construct; identical to SEQ ID NO: 13
  source 1..32: mol_type = other RNA

SEQ ID NO: 37 - RNA, 24 nt, synthetic construct
  source 1..24: mol_type = other RNA
ctggagttcagacgttgtgctctt

SEQ ID NO: 38 - RNA, 32 nt, synthetic construct; identical to SEQ ID NO: 14
  source 1..32: mol_type = other RNA

SEQ ID NO: 39 - RNA, 24 nt, synthetic construct
  source 1..24: mol_type = other RNA
ctggagttcagaccgtgtgctctt

SEQ ID NO: 40 - RNA, 17 nt, synthetic construct
  source 1..17: mol_type = other RNA
gtacattctagatagcc

SEQ ID NO: 41 - RNA, 17 nt, synthetic construct
  source 1..17: mol_type = other RNA
ggctatctagaatgtac

SEQ ID NO: 42 - RNA, 17 nt, synthetic construct
  source 1..17: mol_type = other RNA
gtacattctagatagcc

SEQ ID NO: 43 - RNA, 17 nt, synthetic construct
  source 1..17: mol_type = other RNA
ggctatctagaatgtac

SEQ ID NO: 44 - RNA, 19 nt, synthetic construct
  source 1..19: mol_type = other RNA
ctagaaaactggataacgt

SEQ ID NO: 45 - RNA, 21 nt, synthetic construct
  source 1..21: mol_type = other RNA
acgttatccagttttctagcc

SEQ ID NO: 46 - RNA, 30 nt, synthetic construct
  source 1..30: mol_type = other RNA
ccagagtcgctgagattcgtggcgctatat

SEQ ID NO: 47 - RNA, 32 nt, synthetic construct; identical to SEQ ID NO: 3
  source 1..32: mol_type = other RNA

SEQ ID NO: 48 - RNA, 21 nt, synthetic construct
  source 1..21: mol_type = other RNA
acgttatccagttttctagcc

SEQ ID NO: 49 - RNA, 32 nt, synthetic construct
  source 1..32: mol_type = other RNA
gactggagttcagacgtgtgctcttccgatct

SEQ ID NO: 50 - RNA, 24 nt, synthetic construct
  source 1..24: mol_type = other RNA
gactggagttcagacgtgtgctct

SEQ ID NO: 51 - RNA, 54 nt, synthetic construct
  source 1..54: mol_type = other RNA
  misc_feature 19: note = is linked to Spacer18 at 3' end
ctagaaaactggataacgtgatctggagttcagacgtgttgctcttccgatctc

SEQ ID NO: 52 - RNA, 54 nt, synthetic construct
  source 1..54: mol_type = other RNA
  misc_feature 32: note = is linked to Spacer18 at 3' end
ctggagttcagacgtgttgctcttccgatctcgatctagaaaactggataacgt

SEQ ID NO: 53 - RNA, 53 nt, synthetic construct
  source 1..53: mol_type = other RNA
ctggagttcagacgtgttgctcttccgatctcttctagaaaactggataacgt

SEQ ID NO: 54 - RNA, 53 nt, synthetic construct; identical to SEQ ID NO: 53
  source 1..53: mol_type = other RNA

SEQ ID NO: 55 - RNA, 49 nt, synthetic construct
  source 1..49: mol_type = other RNA
ctggagttcagacgtgttgctcttccgatctcgtacattctagatagcc

SEQ ID NO: 56 - RNA, 51 nt, synthetic construct
  source 1..51: mol_type = other RNA
ctagaaaactggataacgtctggagttcagacgtgttgctcttccgatctc

SEQ ID NO: 57 - RNA, 38 nt, synthetic construct
  source 1..38: mol_type = other RNA
acgttatccagttttctagccggctatctagaatgtac

SEQ ID NO: 58 - RNA, 24 nt, synthetic construct
  source 1..24: mol_type = other RNA
ggacatggattcttgtctgtgtcc

SEQ ID NO: 59 - RNA, 24 nt, synthetic construct
  source 1..24: mol_type = other RNA
gatctgtgtcttagacgtgttgcc

SEQ ID NO: 60 - RNA, 32 nt, synthetic construct
  source 1..32: mol_type = other RNA
gatcgtgacgactcttgtctgctgtcctgatc

SEQ ID NO: 61 - RNA, 32 nt, synthetic construct
  source 1..32: mol_type = other RNA
cgtctccagcatgtgtaggtctctgtctctga

SEQ ID NO: 62 - RNA, 21 nt, synthetic construct
  source 1..21: mol_type = other RNA
ggagttcagacgtgttgctct

SEQ ID NO: 63 - RNA, 26 nt, synthetic construct
  source 1..26: mol_type = other RNA
ctggagttcgttgctcttccgatctc

SEQ ID NO: 64 - RNA, 25 nt, synthetic construct
  source 1..25: mol_type = other RNA
ctggacagacgtgtcttccgatctc

SEQ ID NO: 65 - RNA, 32 nt, synthetic construct
  source 1..32: mol_type = other RNA
ctggagttcagatcagacgtgtgtgttgctct

SEQ ID NO: 66 - RNA, 32 nt, synthetic construct
  source 1..32: mol_type = other RNA
ctggagttcagacgtgtagctcgtgtgatctc

SEQ ID NO: 67 - RNA, 19 nt, synthetic construct
  source 1..19: mol_type = other RNA
cttcttattgacacttaca

SEQ ID NO: 68 - RNA, 19 nt, synthetic construct
  source 1..19: mol_type = other RNA
tgtaagtgtcaataagaag

SEQ ID NO: 69 - RNA, 19 nt, synthetic construct
  source 1..19: mol_type = other RNA
caagaagaatgaatacagt

SEQ ID NO: 70 - RNA, 19 nt, synthetic construct
  source 1..19: mol_type = other RNA
actgtattcattcttcttg

SEQ ID NO: 71 - RNA, 54 nt, synthetic construct; identical to SEQ ID NO: 51
  source 1..54: mol_type = other RNA
  misc_feature 19: note = is linked to Spacer18 at 3' end

SEQ ID NO: 72 - RNA, 53 nt, synthetic construct; identical to SEQ ID NO: 53
  source 1..53: mol_type = other RNA

SEQ ID NO: 73 - RNA, 24 nt, synthetic construct
  source 1..24: mol_type = other RNA
ctggagttcagacgttgtgctctt

SEQ ID NO: 74 - RNA, 24 nt, synthetic construct
  source 1..24: mol_type = other RNA
ctggagttcagacgtgttgctctt

SEQ ID NO: 75 - RNA, 24 nt, synthetic construct
  source 1..24: mol_type = other RNA
ctggagttcagaccgtgtgctctt

SEQ ID NO: 76 - RNA, 21 nt, synthetic construct
  source 1..21: mol_type = other RNA
ctgcttcagacgtgttagctt

SEQ ID NO: 77 - RNA, 24 nt, synthetic construct
  source 1..24: mol_type = other RNA
ggacatggattcttgtctgtgtcc

SEQ ID NO: 78 - RNA, 32 nt, synthetic construct; identical to SEQ ID NO: 61
  source 1..32: mol_type = other RNA

SEQ ID NO: 79 - DNA, 20 bp, synthetic construct
  source 1..20: mol_type = other DNA
cctttggaacgaagggtaca

SEQ ID NO: 80 - DNA, 20 bp, synthetic construct
  source 1..20: mol_type = other DNA
cggactggatctgggtctta

SEQ ID NO: 81 - DNA, 19 bp, synthetic construct
  source 1..19: mol_type = other DNA
ggtcggagtcaacggattt

SEQ ID NO: 82 - DNA, 19 bp, synthetic construct
  source 1..19: mol_type = other DNA
ccagcatcgccccacttga